European Patent Application EP 4 461 743 A2, published November 13, 2024. Title: T cell modification. Applicant: Adaptimmune Limited. The sequence listing filed with the application follows.

SEQUENCE LISTING (18 sequences)

SEQ ID NO: 1 - protein, 235 aa, synthetic construct
  REGION 1..235: note = Synthetic Construct
MALPVTALLLPLALLLHAARPSQFRVSPLDRTWNLGETVELKCQVLLSNPTSGCSWLFQPRGAAASPTFLLYLSQNKPKAAEGLDTQRFSGKRLGDTFVLTLSDFRRENEGYYFCSALSNSIMYFSHFVPVFLPAKPTTTPAPRPPTPAPTIASQPLSLRPEACRPAAGGAVHTRGLDFACDIYIWAPLAGTCGVLLLSLVITLYCNHRNRRRVCKCPRPVVKSGDKPSLSARYV

SEQ ID NO: 2 - DNA, 745 bp, synthetic construct
  misc_feature 1..745: note = Synthetic Construct
  source 1..745: mol_type = other DNA
atggccttaccagtgaccgccttgctcctgccgctggccttgctgctccacgccgccaggccgagccagttccgggtgtcgccgctggatcggacctggaacctgggcgagacagtggagctgaagtgccaggtgctgctgtccaacccgacgtcgggctgctcgtggctcttccagccgcgcggcgccgccgccagtcccaccttcctcctatacctctcccaaaacaagcccaaggcggccgaggggctggacacccagcggttctcgggcaagaggttgggggacaccttcgtcctcaccctgagcgacttccgccgagagaacgagggctactatttctgctcggccctgagcaactccatcatgtacttcagccacttcgtgccggtcttcctgccagcgaagcccaccacgacgccagcgccgcgaccaccaacaccggcgcccaccatcgcgtcgcagcccctgtccctgcgcccagaggcgtgccggccagcggcggggggcgcagtgcacacgagggggctggacttcgcctgtgatatctacatctgggcgcccttggccgggacttgtggggtccttctcctgtcactggttatcaccctttactgcaaccacaggaaccgaagacgtgtttgcaaatgtccccggcctgtggtcaaatcgggagacaagcccagcctttcggcgagatacgtcggttcaagagctaaaagaagtggtagtggtgcccctgtga

SEQ ID NO: 3 - protein, 282 aa, synthetic construct
  REGION 1..282: note = Synthetic Construct
MKKHLTTFLVILWLYFYRGNGKNQVEQSPQSLIILEGKNCTLQCNYTVSPFSNLRWYKQDTGRGPVSLTILTFSENTKSNGRYTATLDADTKQSSLHITASQLSDSASYICVVSGGTDSWGKLQFGAGTQVVVTPDIQNPDPAVYQLRDSKSSDKSVCLFTDFDSQTNVSQSKDSDVYITDKTVLDMRSMDFKSNSAVAWSNKSDFACANAFNNSIIPEDTFFPSPESSCDVKLVEKSFETDTNLNFQNLSVIGFRILLLKVAGFNLLMTLRLWSSGSRAKR

SEQ ID NO: 4 - DNA, 846 bp, synthetic construct
  misc_feature 1..846: note = Synthetic Construct
  source 1..846: mol_type = other DNA
atgaagaagcacctgaccacctttctcgtgatcctgtggctgtacttctaccggggcaacggcaagaaccaggtggaacagagcccccagagcctgatcatcctggaaggcaagaactgcaccctgcagtgcaactacaccgtgtcccccttcagcaacctgcggtggtacaagcaggacaccggcagaggccctgtgtccctgaccatcctgaccttcagcgagaacaccaagagcaacggccggtacaccgccaccctggacgccgatacaaagcagagcagcctgcacatcaccgccagccagctgagcgatagcgccagctacatctgcgtggtgtccggcggcacagacagctggggcaagctgcagtttggcgccggaacacaggtggtcgtgacccccgacatccagaaccctgaccctgccgtgtaccagctgcgggacagcaagagcagcgacaagagcgtgtgcctgttcaccgacttcgacagccagaccaacgtgtcccagagcaaggacagcgacgtgtacatcaccgacaagaccgtgctggacatgcggagcatggacttcaagagcaatagcgccgtggcctggtccaacaagagcgacttcgcctgcgccaacgccttcaacaacagcattatccccgaggacacattcttcccaagccccgagagcagctgcgacgtcaagctggtggaaaagagcttcgagacagacaccaacctgaacttccagaacctgagcgtgatcggcttcagaatcctgctgctgaaggtggccggcttcaacctgctgatgaccctgagactgtggtccagcggcagccgggccaagaga

SEQ ID NO: 5 - protein, 311 aa, synthetic construct
  REGION 1..311: note = Synthetic Construct
MASLLFFCGAFYLLGTGSMDADVTQTPRNRITKTGKRIMLECSQTKGHDRMYWYRQDPGLGLRLIYYSFDVKDINKGEISDGYSVSRQAQAKFSLSLESAIPNQTALYFCATSGQGAYEEQFFGPGTRLTVLEDLKNVFPPEVAVFEPSEAEISHTQKATLVCLATGFYPDHVELSWWVNGKEVHSGVSTDPQPLKEQPALNDSRYCLSSRLRVSATFWQNPRNHFRCQVQFYGLSENDEWTQDRAKPVTQIVSAEAWGRADCGFTSESYQQGVLSATILYEILLGKATLYAVLVSALVLMAMVKRKDSRG

SEQ ID NO: 6 - DNA, 933 bp, synthetic construct
  misc_feature 1..933: note = Synthetic Construct
  source 1..933: mol_type = other DNA
atggccagcctgctgttcttctgcggcgccttctacctgctgggcaccggctctatggatgccgacgtgacccagaccccccggaacagaatcaccaagaccggcaagcggatcatgctggaatgctcccagaccaagggccacgaccggatgtactggtacagacaggaccctggcctgggcctgcggctgatctactacagcttcgacgtgaaggacatcaacaagggcgagatcagcgacggctacagcgtgtccagacaggctcaggccaagttcagcctgtccctggaaagcgccatccccaaccagaccgccctgtacttttgtgccacaagcggccagggcgcctacgaggagcagttctttggccctggcacccggctgacagtgctggaagatctgaagaacgtgttccccccagaggtggccgtgttcgagccttctgaggccgaaatcagccacacccagaaagccacactcgtgtgtctggccaccggcttctaccccgaccacgtggaactgtcttggtgggtcaacggcaaagaggtgcacagcggcgtgtccaccgatccccagcctctgaaagaacagcccgccctgaacgacagccggtactgcctgagcagcagactgagagtgtccgccaccttctggcagaaccccagaaaccacttcagatgccaggtgcagttttacggcctgagcgagaacgacgagtggacccaggacagagccaagcccgtgacacagatcgtgtctgccgaagcttgggggcgcgccgattgtggctttaccagcgagagctaccagcagggcgtgctgagcgccaccatcctgtacgagatcctgctgggaaaggccacactgtacgccgtgctggtgtctgccctggtgctgatggccatggtcaagcggaaggacagccggggc

SEQ ID NO: 7 - protein, 136 aa, synthetic construct
  REGION 1..136: note = Synthetic Construct
MKKHLTTFLVILWLYFYRGNGKNQVEQSPQSLIILEGKNCTLQCNYTVSPFSNLRWYKQDTGRGPVSLTILTFSENTKSNGRYTATLDADTKQSSLHITASQLSDSASYICVVSGGTDSWGKLQFGAGTQVVVTPD

SEQ ID NO: 8 - protein, 133 aa, synthetic construct
  REGION 1..133: note = Synthetic Construct
MASLLFFCGAFYLLGTGSMDADVTQTPRNRITKTGKRIMLECSQTKGHDRMYWYRQDPGLGLRLIYYSFDVKDINKGEISDGYSVSRQAQAKFSLSLESAIPNQTALYFCATSGQGAYEEQFFGPGTRLTVLE

SEQ ID NO: 9 - protein, 6 aa, synthetic construct
  REGION 1..6: note = Synthetic Construct
VSPFSN

SEQ ID NO: 10 - protein, 6 aa, synthetic construct
  REGION 1..6: note = Synthetic Construct
LTFSEN

SEQ ID NO: 11 - protein, 15 aa, synthetic construct
  REGION 1..15: note = Synthetic Construct
CVVSGGTDSWGKLQF

SEQ ID NO: 12 - protein, 5 aa, synthetic construct
  REGION 1..5: note = Synthetic Construct
KGHDR

SEQ ID NO: 13 - protein, 6 aa, synthetic construct
  REGION 1..6: note = Synthetic Construct
SFDVKD

SEQ ID NO: 14 - protein, 14 aa, synthetic construct
  REGION 1..14: note = Synthetic Construct
CATSGQGAYEEQFF

SEQ ID NO: 15 - protein, 9 aa, synthetic construct
  REGION 1..9: note = Synthetic Construct
VLLSNPTSG

SEQ ID NO: 16 - protein, 8 aa, synthetic construct
  REGION 1..8: note = Synthetic Construct
YLSQNKPK

SEQ ID NO: 17 - protein, 6 aa, synthetic construct
  REGION 1..6: note = Synthetic Construct
LSNSIM

SEQ ID NO: 18 - protein, 10 aa, synthetic construct
  REGION 1..10: note = Synthetic Construct
GVYDGREHTV